European Patent Application EP 4 169 947 A1, published April 26, 2023. Title: ANTI-CLAUDIN18.2 ANTIBODY AND USE THEREOF. Applicant: Innovent Biologics (Suzhou) Co., Ltd. The sequence listing filed with the application follows.

SEQUENCE LISTING (94 sequences)

SEQ ID NO: 1 - protein, 10 aa, Artificial
  Synthetic peptide
GFTFSSYVMS

SEQ ID NO: 2 - protein, 17 aa, Artificial
  Synthetic peptide
TISHSGGSTYYADSVKG

SEQ ID NO: 3 - protein, 13 aa, Artificial
  Synthetic peptide
DAPYYDILTGYRY

SEQ ID NO: 4 - protein, 122 aa, Artificial
  Synthetic peptide
EVQLLDSGGGLVQPGGSLRLSCAASGFTFSSYVMSWVRQAPGKGLNWVSTISHSGGSTYYADSVKGRFTISRDNSKNTLYLQMNSLRAEDTAVYYCAIDAPYYDILTGYRYWGQGTLVTVSS

SEQ ID NO: 5 - protein, 330 aa, Artificial
  Synthetic peptide
ASTKGPSVFPLAPSSKSTSGGTAALGCLVKDYFPEPVTVSWNSGALTSGVHTFPAVLQSSGLYSLSSVVTVPSSSLGTQTYICNVNHKPSNTKVDKKAEPKSCDKTHTCPPCPAPELLGGPSVFLFPPKPKDTLMISRTPEVTCVVVDVSHEDPEVKFNWYVDGVEVHNAKTKPREEQYNSTYRVVSVLTVLHQDWLNGKEYKCKVSNKALPAPIEKTISKAKGQPREPQVYTLPPSRDELTKNQVSLTCLVKGFYPSDIAVEWESNGQPENNYKTTPPVLDSDGSFFLYSKLTVDKSRWQQGNVFSCSVMHEALHNHYTQKSLSLSPGK

SEQ ID NO: 6 - protein, 11 aa, Artificial
  Synthetic peptide
RASQSISSWLA

SEQ ID NO: 7 - protein, 7 aa, Artificial
  Synthetic peptide
KASSLES

SEQ ID NO: 8 - protein, 9 aa, Artificial
  Synthetic peptide
QQYNSYSYT

SEQ ID NO: 9 - protein, 107 aa, Artificial
  Synthetic peptide
DIQMTQSPSTLSASVGDRVTITCRASQSISSWLAWYQQKPGKAPKLLIYKASSLESGVPSRFSGSGSGTEFTLTISSLQPDDFATYYCQQYNSYSYTFGQGTKLEIK

SEQ ID NO: 10 - protein, 107 aa, Artificial [sequence omitted]

SEQ ID NO: 11 - protein, 17 aa, Artificial
  Synthetic peptide
  misc_feature (8)..(8): Xaa can be any naturally occurring amino acid
KSSQSLLXGGNQKNYLT

SEQ ID NO: 12 - protein, 10 aa, Artificial
  Synthetic peptide
GYSFSSYNIH

SEQ ID NO: 13 - protein, 17 aa, Artificial
  Synthetic peptide
YIAPFNGDSRYNQKFKG

SEQ ID NO: 14 - protein, 9 aa, Artificial
  Synthetic peptide
LNRGNSLDY

SEQ ID NO: 15 - protein, 118 aa, Artificial
  Synthetic peptide
EVQLQQSGPELMKPGASVKISCKATGYSFSSYNIHWVKQSHGKSLEWIGYIAPFNGDSRYNQKFKGKATVTVDKSSSTAYMHLSSLTSEDSAVYYCGRLNRGNSLDYWGQGTSLTVSS

SEQ ID NO: 16 - protein, 17 aa, Artificial
  Synthetic peptide
KSSQSLFNSGNQRNYLT

SEQ ID NO: 17 - protein, 7 aa, Artificial
  Synthetic peptide
WASTRES

SEQ ID NO: 18 - protein, 9 aa, Artificial
  Synthetic peptide
QNNYIYPLT

SEQ ID NO: 19 - protein, 113 aa, Artificial
  Synthetic peptide
DIVMTQSPSSLTVTAGEKVTMSCKSSQSLFNSGNQRNYLTWYQQKPGQPPKLLIYWASTRESGVPDRFTGSGSGTDFTLTISSVQAEDLAFYYCQNNYIYPLTFGAGTKLELK

SEQ ID NO: 20 - protein, 17 aa, Artificial
  Synthetic peptide
YIAPFQGDSRYNQKFKG

SEQ ID NO: 21 - protein, 118 aa, Artificial
  Synthetic peptide
QVQLVQSGAEVKKPGSSVKVSCKASGYSFSSYNIHWVRQAPGQGLEWMGYIAPFQGDSRYNQKFKGRVTITADKSTSTAYMELSSLRSEDTAVYYCARLNRGNSLDYWGQGTLVTVSS

SEQ ID NO: 22 - protein, 113 aa, Artificial
  Synthetic peptide
DIVMTQSPDSLAVSLGERATINCKSSQSLFNSGNQRNYLTWYQQKPGQPPKLLIYWASTRESGVPDRFSGSGSGTDFTLTISSLQAEDVAVYYCQNNYIYPLTFGGGTKVEIK

SEQ ID NO: 23 - protein, 10 aa, Artificial
  Synthetic peptide
GFSFSDYGMH

SEQ ID NO: 24 - protein, 17 aa, Artificial
  Synthetic peptide
YINSGSRTLYYADTVKG

SEQ ID NO: 25 - protein, 10 aa, Artificial
  Synthetic peptide
NAYYGNAMDY

SEQ ID NO: 26 - protein, 119 aa, Artificial
  Synthetic peptide
EVQLVESGGGLVKPGGSLKLSCAASGFSFSDYGMHWVRQAPEKGLEWIAYINSGSRTLYYADTVKGRFTISRDNAKNTLFLQMTSLRSEETAMYYCTRNAYYGNAMDYWGQGTSVTVSS

SEQ ID NO: 27 - protein, 119 aa, Artificial
  Synthetic peptide
EVQLVESGGGLVQPGGSLRLSCAASGFSFSDYGMHWVRQAPGKGLEWVSYINSGSRTLYYADTVKGRFTISRDNAKNSLYLQMNSLRDEDTAVYYCARNAYYGNAMDYWGQGTLVTVSS

SEQ ID NO: 28 - protein, 17 aa, Artificial
  Synthetic peptide
KSSQSLLNSGNQRNYLT

SEQ ID NO: 29 - protein, 7 aa, Artificial
  Synthetic peptide
WSSTRGS

SEQ ID NO: 30 - protein, 9 aa, Artificial
  Synthetic peptide
QNVYYYPFT

SEQ ID NO: 31 - protein, 113 aa, Artificial
  Synthetic peptide
DIQMTQSPSSLTVTAGEKVTMSCKSSQSLLNSGNQRNYLTWYQQIPGQPPKLLIYWSSTRGSGVPDRFTGSGSGTDFTLTISSVQAEDLAVYFCQNVYYYPFTFGSGTRLEVK

SEQ ID NO: 32 - protein, 113 aa, Artificial
  Synthetic peptide
DIVMTQSPDSLAVSLGERATINCKSSQSLLNSGNQRNYLTWYQQKPGQPPKLLIYWSSTRGSGVPDRFSGSGSGTDFTLTISSLQAEDVAVYYCQNVYYYPFTFGQGTRLEIK

SEQ ID NO: 33 - protein, 11 aa, Artificial
  Synthetic peptide
GYSITSGYGWN

SEQ ID NO: 34 - protein, 16 aa, Artificial
  Synthetic peptide
YIHFSGSTNYNPSLKS

SEQ ID NO: 35 - protein, 9 aa, Artificial
  Synthetic peptide
SGKGNAMDY

SEQ ID NO: 36 - protein, 118 aa, Artificial
  Synthetic peptide
QVQLKESGPDLVKPSQSLSLTCTVTGYSITSGYGWNWIRQFPGNKLEWMGYIHFSGSTNYNPSLKSRISITRDTSKNQFFLQLNSVTTEDTATYYCARSGKGNAMDYWGQGTSVTVSS

SEQ ID NO: 37 - protein, 118 aa, Artificial
  Synthetic peptide
QVQLQESGPGLVKPSETLSLTCTVSGYSITSGYGWNWIRQPPGKGLEWIGYIHFSGSTNYNPSLKSRVTISVDTSKNQFSLKLSSVTAADTAVYYCARSGKGNAMDYWGQGTLVTVSS

SEQ ID NO: 38 - protein, 17 aa, Artificial
  Synthetic peptide
KSSQSLLNSGNQKNYLT

SEQ ID NO: 39 - protein, 9 aa, Artificial
  Synthetic peptide
QNDYYFPFT

SEQ ID NO: 40 - protein, 113 aa, Artificial
  Synthetic peptide
DIQMTQSPSSLTVTAGEKVTMSCKSSQSLLNSGNQKNYLTWYQQKPGQPPKLLIYWASTRESGVPDRFTGSGSGTDFTLTVINMQAEDLALYYCQNDYYFPFTFGSGTKLEIK

SEQ ID NO: 41 - protein, 113 aa, Artificial
  Synthetic peptide
DIVMTQSPDSLAVSLGERATINCKSSQSLLNSGNQKNYLTWYQQKPGQPPKLLIYWASTRESGVPDRFSGSGSGTDFTLTISSLQAEDVAVYYCQNDYYFPFTFGGGTKVEIK

SEQ ID NO: 42 - protein, 10 aa, Artificial
  Synthetic peptide
GYTFTKYIIQ

SEQ ID NO: 43 - protein, 17 aa, Artificial
  Synthetic peptide
YINPYNDDTKYNEKFKG

SEQ ID NO: 44 - protein, 9 aa, Artificial
  Synthetic peptide
TYYGNSFPN

SEQ ID NO: 45 - protein, 118 aa, Artificial
  Synthetic peptide
EVQLQQSVPELVKPGASVRMSCKASGYTFTKYIIQWVKQKPGQGLEWIAYINPYNDDTKYNEKFKGKATLTSDKSASTAYMELSSLTSEDSAVYYCATTYYGNSFPNWGQGTLVTVSA

SEQ ID NO: 46 - protein, 9 aa, Artificial
  Synthetic peptide
QNDYSFPFT

SEQ ID NO: 47 - protein, 113 aa, Artificial
  Synthetic peptide
DIVMTQSPSSLTVTAGERVTMTCKSSQSLLNSGNQKNYLTWYQQKPGQPPKLLIYWASTRESGVPDRFTGSGSGTDFTLTISSLQSEDLAVYFCQNDYSFPFTFGSGTKLEIK

SEQ ID NO: 48 - protein, 118 aa, Artificial
  Synthetic peptide
QVQLVQSGAEVKKPGASVKVSCKASGYTFTKYIIQWVRQAPGQRLEWMGYINPYNDDTKYNEKFKGRVTITRDTSASTAYMELSSLRSEDMAVYYCARTYYGNSFPNWGQGTLVTVSS

SEQ ID NO: 49 - protein, 113 aa, Artificial
  Synthetic peptide
DIVMTQSPDSLAVSLGERATINCKSSQSLLNSGNQKNYLTWYQQKPGQPPKLLIYWASTRESGVPDRFSGSGSGTDFTLTISSLQAEDVAVYYCQNDYSFPFTFGGGTKVEIK

SEQ ID NO: 50 - protein, 10 aa, Artificial
  Synthetic peptide
GFSLTDYGVS

SEQ ID NO: 51 - protein, 16 aa, Artificial
  Synthetic peptide
VMWGGGNTYYNSALKS

SEQ ID NO: 52 - protein, 10 aa, Artificial
  Synthetic peptide
QRYGGNAMDY

SEQ ID NO: 53 - protein, 118 aa, Artificial
  Synthetic peptide
QVQLKESGPGLVAPSQSLSITCTVSGFSLTDYGVSWIRQPPGKGLEWLGVMWGGGNTYYNSALKSRLSISKDNSKSQVFLKMNSLQSDDTAMYYCAKQRYGGNAMDYWGQGTSVTVSS

SEQ ID NO: 54 - protein, 9 aa, Artificial
  Synthetic peptide
QNSYFYPFT

SEQ ID NO: 55 - protein, 113 aa, Artificial
  Synthetic peptide
DIQMTQSPSSLTVTAGEKVTMSCKSSQSLLNSGNQRNYLTWYQQIPGQPPKLLIYWASTRESGVPNRFTGSGSGAEFTLTISSVQTEDLAVYYCQNSYFYPFTFGAGTKLELK

SEQ ID NO: 56 - protein, 118 aa, Artificial
  Synthetic peptide
QVQLQESGPGLVKPSETLSLTCTVSGFSLTDYGVSWIRQPPGKGLEWIGVMWGGGNTYYNSALKSRVTISVDTSKNQFSLKLSSVTAADTAVYYCARQRYGGNAMDYWGQGTLVTVSS

SEQ ID NO: 57 - protein, 113 aa, Artificial
  Synthetic peptide
DIVMTQSPDSLAVSLGERATINCKSSQSLLNSGNQRNYLTWYQQKPGQPPKLLIYWASTRESGVPDRFSGSGSGTDFTLTISSLQAEDVAVYYCQNSYFYPFTFGGGTKVEIK

SEQ ID NO: 58 - protein, 10 aa, Artificial
  Synthetic peptide
GFTFSDYGMA

SEQ ID NO: 59 - protein, 17 aa, Artificial
  Synthetic peptide
FINNLAYSIYYVDTVTG

SEQ ID NO: 60 - protein, 9 aa, Artificial
  Synthetic peptide
FTTGNVMDY

SEQ ID NO: 61 - protein, 118 aa, Artificial
  Synthetic peptide
EVMLVESGGGLVQPGGSRKLSCAASGFTFSDYGMAWVRQAPGKGPEWVAFINNLAYSIYYVDTVTGRFTISRENAKDTLYLEMSSLRSEDTALYYCARFTTGNVMDYWGQGTSVTVSS

SEQ ID NO: 62 - protein, 17 aa, Artificial
  Synthetic peptide
KSSQSLLNGGNQKNYLT

SEQ ID NO: 63 - protein, 7 aa, Artificial
  Synthetic peptide
WSSTRES

SEQ ID NO: 64 - protein, 9 aa, Artificial
  Synthetic peptide
QNSYSYPLT

SEQ ID NO: 65 - protein, 113 aa, Artificial
  Synthetic peptide
DIVMTQSPSSLTVTAGEKVTMTCKSSQSLLNGGNQKNYLTWYQQKPGQPPKLLIYWSSTRESGVPDRFTGSGSGTDFTLTITSVQAEDLAVYYCQNSYSYPLTFGSGTKLELK

SEQ ID NO: 66 - protein, 118 aa, Artificial
  Synthetic peptide
EVQLVESGGGLVQPGGSLRLSCAASGFTFSDYGMAWVRQAPGKGLEWVAFINNLAYSIYYVDTVTGRFTISRDNAKNSLYLQMNSLRAEDTAVYYCARFTTGNVMDYWGQGTLVTVSS

SEQ ID NO: 67 - protein, 17 aa, Artificial
  Synthetic peptide
KSSQSLLQGGNQKNYLT

SEQ ID NO: 68 - protein, 113 aa, Artificial
  Synthetic peptide
DIVMTQSPDSLAVSLGERATINCKSSQSLLQGGNQKNYLTWYQQKPGQPPKLLIYWSSTRESGVPDRFSGSGSGTDFTLTISSLQAEDVAVYYCQNSYSYPLTFGGGTKVEIK

SEQ ID NO: 69 - protein, 10 aa, Artificial
  Synthetic peptide
GYSFTTYWMH

SEQ ID NO: 70 - protein, 17 aa, Artificial
  Synthetic peptide
LIDPSDSETRLNQKFKD

SEQ ID NO: 71 - protein, 6 aa, Artificial
  Synthetic peptide
NRWLLG

SEQ ID NO: 72 - protein, 115 aa, Artificial
  Synthetic peptide
QVQLQQSGPQLVRPGASVKISCKASGYSFTTYWMHWVKQRPGQGLEWIGLIDPSDSETRLNQKFKDKATLTVDKSSSTAYMRLSSPTSEDSAVYYCASNRWLLGWGQGTLVTVSS

SEQ ID NO: 73 - protein, 115 aa, Artificial
  Synthetic peptide
QVQLVQSGAEVKKPGASVKVSCKASGYSFTTYWMHWVRQAPGQGLEWMGLIDPSDSETRLNQKFKDRVTMTVDTSTSTVYMELSSLRSEDTAVYYCASNRWLLGWGQGTLVTVSS

SEQ ID NO: 74 - protein, 9 aa, Artificial
  Synthetic peptide
QNDYSYPLT

SEQ ID NO: 75 - protein, 113 aa, Artificial
  Synthetic peptide
DIQMIQSPSSLTVTAGEKVTMSCKSSQSLLNSGNQKNYLTWYQQKPGQPPKLLIYWASTRESGVPDRFTGSGSGTDFTLTISSVQTEDLAVYYCQNDYSYPLTFGAGTKLEIK

SEQ ID NO: 76 - protein, 113 aa, Artificial
  Synthetic peptide
DIVMTQSPDSLAVSLGERATINCKSSQSLLNSGNQKNYLTWYQQKPGQPPKLLIYWASTRESGVPDRFSGSGSGTDFTLTISSLQAEDVAVYYCQNDYSYPLTFGQGTKLEIK

SEQ ID NO: 77 - protein, 10 aa, Artificial
  Synthetic peptide
GFSLNSYGVG

SEQ ID NO: 78 - protein, 16 aa, Artificial
  Synthetic peptide
VIWGDGSTNYHSVLIS

SEQ ID NO: 79 - protein, 9 aa, Artificial
  Synthetic peptide
ITRGNAMDY

SEQ ID NO: 80 - protein, 117 aa, Artificial
  Synthetic peptide
QVQLKESGPGLVAPSQSLSITCSVSGFSLNSYGVGWVRQPPGKGLEWLGVIWGDGSTNYHSVLISRLSIRKDNSKSQVFLKLNSLQTDDTATYYCAMITRGNAMDYWGQGTSVTVSS

SEQ ID NO: 81 - protein, 7 aa, Artificial
  Synthetic peptide
WASTRKS

SEQ ID NO: 82 - protein, 9 aa, Artificial
  Synthetic peptide
QNNYLFPLT

SEQ ID NO: 83 - protein, 113 aa, Artificial
  Synthetic peptide
DIVMTQSPSSLTVTAGEKITMSCKSSQSLLNSGNQRNYLTWYQQKPGQTPKLLIYWASTRKSGVPDRFTGSGSGTDFTLTISSVQAEDLAVYSCQNNYLFPLTFGAGTKLELK

SEQ ID NO: 84 - protein, 16 aa, Artificial
  Synthetic peptide
VIWGDVSTNYHSVLIS

SEQ ID NO: 85 - protein, 117 aa, Artificial
  Synthetic peptide
QVQLQESGPGLVKPSETLSLTCTVSGFSLNSYGVGWIRQPPGKGLEWIGVIWGDVSTNYHSVLISRVTISKDTSKNQVSLKLSSVTAADTAVYYCARITRGNAMDYWGQGTLVTVSS

SEQ ID NO: 86 - protein, 113 aa, Artificial
  Synthetic peptide
DIVMTQSPDSLAVSLGERATINCKSSQSLLNSGNQRNYLTWYQQKPGQPPKLLIYWASTRKSGVPDRFSGSGSGTDFTLTISSLQAEDVAVYYCQNNYLFPLTFGGGTKVEIK

SEQ ID NO: 87 - protein, 10 aa, Artificial
  Synthetic peptide
GYTFTSYWIN

SEQ ID NO: 88 - protein, 16 aa, Artificial
  Synthetic peptide
NIYPSDSYTNYNQKFK

SEQ ID NO: 89 - protein, 9 aa, Artificial
  Synthetic peptide
SWRGNSFDY

SEQ ID NO: 90 - protein, 118 aa, Artificial
  Synthetic peptide
QVQLQQPGAELVRPGASVKLSCKASGYTFTSYWINWVKQRPGQGLEWIGNIYPSDSYTNYNQKFKDKATLTVDKSSSTAYMQLSSPTSEDSAVYYCTRSWRGNSFDYWGQGTTLTVSS

SEQ ID NO: 91 - protein, 9 aa, Artificial
  Synthetic peptide
QNDYSYPFT

SEQ ID NO: 92 - protein, 113 aa, Artificial
  Synthetic peptide
DIVMTQSPSSLTVTAGEKVTMSCKSSQSLLNSGNQKNYLTWYQQKPGQPPKLLIYWASTRESGVPDRFTGSGSGTDFTLTISSVQAEDLAVYYCQNDYSYPFTFGSGTKLEIK

SEQ ID NO: 93 - protein, 17 aa, Artificial
  Synthetic peptide
  misc_feature (6)..(6): Xaa can be any naturally occurring amino acid
YIAPFXGDSRYNQKFKG

SEQ ID NO: 94 - protein, 16 aa, Artificial
  Synthetic peptide
  misc_feature (6)..(6): Xaa can be any naturally occurring amino acid
VIWGDXSTNYHSVLIS